European Patent Specification EP 3 143 036 B1, published August 2, 2023. Title: PAR-1 BASED THERAPEUTIC CONJUGATES AND USES THEREOF. Applicant: Tel Hashomer Medical Research Infrastructure and Services Ltd. The sequence listing filed with the application follows.

SEQUENCE LISTING (19 sequences)

SEQ ID NO: 1 - protein, 4 aa, Artificial sequence
  Peptide
LDPR

SEQ ID NO: 2 - protein, 5 aa, Artificial sequence
  Peptide
TLDPR

SEQ ID NO: 3 - protein, 6 aa, Artificial sequence
  Peptide
ATLDPR

SEQ ID NO: 4 - protein, 7 aa, Artificial sequence
  Peptide
NATLDPR

SEQ ID NO: 5 - protein, 8 aa, Artificial sequence
  Peptide
TNATLDPR

SEQ ID NO: 6 - protein, 9 aa, Artificial sequence
  Peptide
ATNATLDPR

SEQ ID NO: 7 - protein, 10 aa, Artificial sequence
  Peptide
KATNATLDPR

SEQ ID NO: 8 - protein, 11 aa, Artificial sequence
  Peptide
SKATNATLDPR

SEQ ID NO: 9 - protein, 12 aa, Artificial sequence
  Peptide
ESKATNATLDPR

SEQ ID NO: 10 - protein, 13 aa, Artificial sequence
  Peptide
PESKATNATLDPR

SEQ ID NO: 11 - protein, 14 aa, Artificial sequence
  Peptide
RPESKATNATLDPR

SEQ ID NO: 12 - protein, 15 aa, Artificial sequence
  Peptide
RRPESKATNATLDPR

SEQ ID NO: 13 - protein, 16 aa, Artificial sequence
  Peptide
ARRPESKATNATLDPR

SEQ ID NO: 14 - protein, 17 aa, Artificial sequence
  Peptide
RARRPESKATNATLDPR

SEQ ID NO: 15 - protein, 18 aa, Artificial sequence
  Peptide
TRARRPESKATNATLDPR

SEQ ID NO: 16 - protein, 19 aa, Artificial sequence
  Peptide
RTRARRPESKATNATLDPR

SEQ ID NO: 17 - protein, 18 aa, Artificial sequence
  Peptide
LDPRSFLLRNPNDKYEPF

SEQ ID NO: 18 - protein, 18 aa, Artificial sequence
  Peptide
LDPRSFLLRNPNDKYEPF

SEQ ID NO: 19 - protein, 5 aa, Artificial sequence
  Peptide
KYEPF